European Patent Specification EP 3 239 169 B1, published April 17, 2024. Title: CONOTOXIN PEPTIDE κ-CPTX-BTL05, PREPARATION METHOD THEREFOR, AND USES THEREOF. Applicant: BGI SHEN ZHEN CO., LIMITED. The sequence listing filed with the application follows.

SEQUENCE LISTING (2 sequences)

SEQ ID NO: 1 - protein, 16 aa, artificial sequence
GICCVDDTCTTHSGCL

SEQ ID NO: 2 - DNA, 48 bp, artificial sequence
ggcatctgctgtgtggatgatacttgtaccacccactcgggatgtctg